European Patent Application EP 4 492 387 A2, published January 15, 2025. Title: COMPUTER-IMPLEMENTED METHODS AND SYSTEMS FOR TRANSCRIPTOMICS. Applicant: Diagenode S.A. Application EP 22768668.0, filed August 19, 2022. The sequence listing filed with the application follows.

SEQUENCE LISTING (1 sequence)

SEQ ID NO: 1 - DNA, 43 bp, synthetic construct
  source 1..43: mol_type = other DNA
agatcggaagagcacacgtctgaaaaaaaagaactccagtcac